European Patent Application EP 4 556 010 A2, published May 21, 2025. Title: ANTIVIRAL JAK INHIBITORS USEFUL IN TREATING OR PREVENTING RETROVIRAL AND OTHER VIRAL INFECTIONS. Applicant: Emory University. Application EP 25154263.5, filed January 27, 2025. The sequence listing filed with the application follows.

SEQUENCE LISTING (7 sequences)

SEQ ID NO: 1 - DNA, 24 bp, synthetic construct
  source 1..24: mol_type = other DNA; note = CpG ODN 7909
tcgtcgttttgtcgttttgtcgtt

SEQ ID NO: 2 - DNA, 17 bp, synthetic construct
  source 1..17: mol_type = other DNA; note = COXII sense primer
tgcccgccatcatccta

SEQ ID NO: 3 - DNA, 21 bp, synthetic construct
  source 1..21: mol_type = other DNA; note = COXII probe
  misc_feature <1: note = 5'-tetrachloro-6-carboxyfluorescein
  misc_feature >21: note = 3'-TAMRA
tcctcatcgccctcccatccc

SEQ ID NO: 4 - DNA, 23 bp, synthetic construct
  source 1..23: mol_type = other DNA; note = COXII antisense primer
cgtctgttatgtaaaggatgcgt

SEQ ID NO: 5 - DNA, 17 bp, synthetic construct
  source 1..17: mol_type = other DNA; note = Beta-actin exon 3 sense primer
gcgcggctacagcttca

SEQ ID NO: 6 - DNA, 18 bp, synthetic construct
  source 1..18: mol_type = other DNA; note = Beta-actin exon 3 probe
  misc_feature <1: note = 5'-6-FAM
  misc_feature >18: note = 3'-TAMRA
caccacggccgagcggga

SEQ ID NO: 7 - DNA, 22 bp, synthetic construct
  source 1..22: mol_type = other DNA; note = Beta-actin exon 3 antisense primer
tctccttaatgtcacgcacgat